European Patent Application EP 4 124 344 A1, published February 1, 2023. Title: Novel use of Hic-5 inhibitor. Applicant: Showa University. The sequence listing filed with the application follows.

SEQUENCE LISTING (31 sequences)

SEQ ID NO: 1 - DNA, 1805 bp, Homo sapiens
  CDS (38)..(1423)
gccctgttcgccccgcgccaccggcccgcgccccgccatggaggacctggatgccctgctctctgacctggagactaccacctcgcacatgccaaggtcaggggctcccaaagagcgccctgcggagcctctcacccctcccccatcctatggccaccagccacagacagggtctggggagtcttcaggagcctcgggggacaaggaccacctgtacagcacggtatgcaagcctcggtccccaaagcctgcagccccggcggcccctccattctcctcttccagcggtgtcttgggtaccgggctctgtgagctagatcggttgcttcaggaacttaatgccactcagttcaacatcacagatgaaatcatgtctcagttcccatctagcaaggtggcttcaggagagcagaaggaggaccagtctgaagataagaaaagacccagcctcccttccagcccgtctcctggcctcccaaaggcttctgccacctcagccactctggagctggatagactgatggcctcactctctgacttccgcgttcaaaaccatcttccagcctctgggccaactcagccaccggtggtgagctccacaaatgagggctccccatccccaccagagccgactggcaagggcagcctagacaccatgctggggctgctgcagtccgacctcagccgccggggtgttcccacccaggccaaaggcctctgtggctcctgcaataaacctattgctgggcaagtggtgacggctctgggccgcgcctggcaccccgagcacttcgtttgcggaggctgttccaccgccctgggaggcagcagcttcttcgagaaggatggagcccccttctgccccgagtgctactttgagcgcttctcgccaagatgtggcttctgcaaccagcccatccgacacaagatggtgaccgccttgggcactcactggcacccagagcatttctgctgcgtcagttgcggggagcccttcggagatgagggtttccacgagcgcgagggccgcccctactgccgccgggacttcctgcagctgttcgccccgcgctgccagggctgccagggccccatcctggataactacatctcggcgctcagcgcgctctggcacccggactgtttcgtctgcagggaatgcttcgcgcccttctcgggaggcagctttttcgagcacgagggccgcccgttgtgcgagaaccacttccacgcacgacgcggctcgctgtgcgccacgtgtggcctccctgtgaccggccgctgcgtgtcggccctgggtcgccgcttccacccggaccacttcacatgcaccttctgcctgcgcccgctcaccaaggggtccttccaggagcgcgccggcaagccctactgccagccctgcttcctgaagctcttcggctgacagcccgctcggctcgccctctcccccggaggccgcgccctcccggaaaagccgggtcctccagaccccgaggccttgctctcagagcgggaggccccacccactggagagccccgcccctaaggtactatgagtcctcaggggtcaagttcagaaacggcccagccagacctaaacccacacgcccacaaagtggattgcacacagacaagaactcccgtgcgggcctccactctattcccacccttgagggagcccccttactgggggagggtccttgcaattccagcgaatcggaggccaggccaggacgtccttgctccctgcaccctcactgttctgtgcactttttctacctacataaacacacgcattccacctc

SEQ ID NO: 2 - protein, 461 aa, Homo sapiens
MEDLDALLSDLETTTSHMPRSGAPKERPAEPLTPPPSYGHQPQTGSGESSGASGDKDHLYSTVCKPRSPKPAAPAAPPFSSSSGVLGTGLCELDRLLQELNATQFNITDEIMSQFPSSKVASGEQKEDQSEDKKRPSLPSSPSPGLPKASATSATLELDRLMASLSDFRVQNHLPASGPTQPPVVSSTNEGSPSPPEPTGKGSLDTMLGLLQSDLSRRGVPTQAKGLCGSCNKPIAGQVVTALGRAWHPEHFVCGGCSTALGGSSFFEKDGAPFCPECYFERFSPRCGFCNQPIRHKMVTALGTHWHPEHFCCVSCGEPFGDEGFHEREGRPYCRRDFLQLFAPRCQGCQGPILDNYISALSALWHPDCFVCRECFAPFSGGSFFEHEGRPLCENHFHARRGSLCATCGLPVTGRCVSALGRRFHPDHFTCTFCLRPLTKGSFQERAGKPYCQPCFLKLFG

SEQ ID NO: 3 - DNA, 1812 bp, Homo sapiens
  CDS (85)..(1419)
ggagaataaaataatcaggaggctgggtttgtgcttggctccaagcatgccctgctctctgacctggagactaccacctcgcacatgccaaggtcaggggctcccaaagagcgccctgcggagcctctcacccctcccccatcctatggccaccagccacagacagggtctggggagtcttcaggagcctcgggggacaaggaccacctgtacagcacggtatgcaagcctcggtccccaaagcctgcagccccggcggcccctccattctcctcttccagcggtgtcttgggtaccgggctctgtgagctagatcggttgcttcaggaacttaatgccactcagttcaacatcacagatgaaatcatgtctcagttcccatctagcaaggtggcttcaggagagcagaaggaggaccagtctgaagataagaaaagacccagcctcccttccagcccgtctcctggcctcccaaaggcttctgccacctcagccactctggagctggatagactgatggcctcactctctgacttccgcgttcaaaaccatcttccagcctctgggccaactcagccaccggtggtgagctccacaaatgagggctccccatccccaccagagccgactggcaagggcagcctagacaccatgctggggctgctgcagtccgacctcagccgccggggtgttcccacccaggccaaaggcctctgtggctcctgcaataaacctattgctgggcaagtggtgacggctctgggccgcgcctggcaccccgagcacttcgtttgcggaggctgttccaccgccctgggaggcagcagcttcttcgagaaggatggagcccccttctgccccgagtgctactttgagcgcttctcgccaagatgtggcttctgcaaccagcccatccgacacaagatggtgaccgccttgggcactcactggcacccagagcatttctgctgcgtcagttgcggggagcccttcggagatgagggtttccacgagcgcgagggccgcccctactgccgccgggacttcctgcagctgttcgccccgcgctgccagggctgccagggccccatcctggataactacatctcggcgctcagcgcgctctggcacccggactgtttcgtctgcagggaatgcttcgcgcccttctcgggaggcagctttttcgagcacgagggccgcccgttgtgcgagaaccacttccacgcacgacgcggctcgctgtgcgccacgtgtggcctccctgtgaccggccgctgcgtgtcggccctgggtcgccgcttccacccggaccacttcacatgcaccttctgcctgcgcccgctcaccaaggggtccttccaggagcgcgccggcaagccctactgccagccctgcttcctgaagctcttcggctgacagcccgctcggctcgccctctcccccggaggccgcgccctcccggaaaagccgggtcctccagaccccgaggccttgctctcagagcgggaggccccacccactggagagccccgcccctaaggtactatgagtcctcaggggtcaagttcagaaacggcccagccagacctaaacccacacgcccacaaagtggattgcacacagacaagaactcccgtgcgggcctccactctattcccacccttgagggagcccccttactgggggagggtccttgcaattccagcgaatcggaggccaggccaggacgtccttgctccctgcaccctcactgttctgtgcactttttctacctacataaacacacgcattccacctctcaaaaaaaaa

SEQ ID NO: 4 - protein, 444 aa, Homo sapiens
MPRSGAPKERPAEPLTPPPSYGHQPQTGSGESSGASGDKDHLYSTVCKPRSPKPAAPAAPPFSSSSGVLGTGLCELDRLLQELNATQFNITDEIMSQFPSSKVASGEQKEDQSEDKKRPSLPSSPSPGLPKASATSATLELDRLMASLSDFRVQNHLPASGPTQPPVVSSTNEGSPSPPEPTGKGSLDTMLGLLQSDLSRRGVPTQAKGLCGSCNKPIAGQVVTALGRAWHPEHFVCGGCSTALGGSSFFEKDGAPFCPECYFERFSPRCGFCNQPIRHKMVTALGTHWHPEHFCCVSCGEPFGDEGFHEREGRPYCRRDFLQLFAPRCQGCQGPILDNYISALSALWHPDCFVCRECFAPFSGGSFFEHEGRPLCENHFHARRGSLCATCGLPVTGRCVSALGRRFHPDHFTCTFCLRPLTKGSFQERAGKPYCQPCFLKLFG

SEQ ID NO: 5 - DNA, 1782 bp, Homo sapiens
  CDS (55)..(1389)
ggggccggatccccggatgccctgctctctgacctggagactaccacctcgcacatgccaaggtcaggggctcccaaagagcgccctgcggagcctctcacccctcccccatcctatggccaccagccacagacagggtctggggagtcttcaggagcctcgggggacaaggaccacctgtacagcacggtatgcaagcctcggtccccaaagcctgcagccccggcggcccctccattctcctcttccagcggtgtcttgggtaccgggctctgtgagctagatcggttgcttcaggaacttaatgccactcagttcaacatcacagatgaaatcatgtctcagttcccatctagcaaggtggcttcaggagagcagaaggaggaccagtctgaagataagaaaagacccagcctcccttccagcccgtctcctggcctcccaaaggcttctgccacctcagccactctggagctggatagactgatggcctcactctctgacttccgcgttcaaaaccatcttccagcctctgggccaactcagccaccggtggtgagctccacaaatgagggctccccatccccaccagagccgactggcaagggcagcctagacaccatgctggggctgctgcagtccgacctcagccgccggggtgttcccacccaggccaaaggcctctgtggctcctgcaataaacctattgctgggcaagtggtgacggctctgggccgcgcctggcaccccgagcacttcgtttgcggaggctgttccaccgccctgggaggcagcagcttcttcgagaaggatggagcccccttctgccccgagtgctactttgagcgcttctcgccaagatgtggcttctgcaaccagcccatccgacacaagatggtgaccgccttgggcactcactggcacccagagcatttctgctgcgtcagttgcggggagcccttcggagatgagggtttccacgagcgcgagggccgcccctactgccgccgggacttcctgcagctgttcgccccgcgctgccagggctgccagggccccatcctggataactacatctcggcgctcagcgcgctctggcacccggactgtttcgtctgcagggaatgcttcgcgcccttctcgggaggcagctttttcgagcacgagggccgcccgttgtgcgagaaccacttccacgcacgacgcggctcgctgtgcgccacgtgtggcctccctgtgaccggccgctgcgtgtcggccctgggtcgccgcttccacccggaccacttcacatgcaccttctgcctgcgcccgctcaccaaggggtccttccaggagcgcgccggcaagccctactgccagccctgcttcctgaagctcttcggctgacagcccgctcggctcgccctctcccccggaggccgcgccctcccggaaaagccgggtcctccagaccccgaggccttgctctcagagcgggaggccccacccactggagagccccgcccctaaggtactatgagtcctcaggggtcaagttcagaaacggcccagccagacctaaacccacacgcccacaaagtggattgcacacagacaagaactcccgtgcgggcctccactctattcccacccttgagggagcccccttactgggggagggtccttgcaattccagcgaatcggaggccaggccaggacgtccttgctccctgcaccctcactgttctgtgcactttttctacctacataaacacacgcattccacctctcaaaaaaaaa

SEQ ID NO: 6 - protein, 444 aa, Homo sapiens; identical to SEQ ID NO: 4

SEQ ID NO: 7 - RNA, 19 nt, Artificial
  Synthetic oligonucleotide
ucugugagcuagaccguuu

SEQ ID NO: 8 - RNA, 20 nt, Artificial
  Synthetic oligonucleotide
gggaaugccuugcgccccuu

SEQ ID NO: 9 - RNA, 19 nt, Artificial
  Synthetic oligonucleotide
agugcuacuuugagcgcuu

SEQ ID NO: 10 - RNA, 19 nt, Artificial
  Synthetic oligonucleotide
gggacaaggaucaucuaua

SEQ ID NO: 11 - RNA, 19 nt, Artificial
  Synthetic oligonucleotide
ccuugcaauuccagcgaau

SEQ ID NO: 12 - RNA, 19 nt, Artificial
  Synthetic oligonucleotide
ggagcuggauagacugaug

SEQ ID NO: 13 - RNA, 19 nt, Artificial
  Synthetic oligonucleotide
caucagucuauccagcucc

SEQ ID NO: 14 - RNA, 19 nt, Artificial
  Synthetic oligonucleotide
ggaccagucugaagauaag

SEQ ID NO: 15 - RNA, 21 nt, Artificial
  Synthetic oligonucleotide
ggagcuggauagacugauguu

SEQ ID NO: 16 - RNA, 21 nt, Artificial
  Synthetic oligonucleotide
ggaccagucugaagauaaguu

SEQ ID NO: 17 - DNA, 19 bp, Homo sapiens
gcagcagcttcttcgagaa

SEQ ID NO: 18 - DNA, 21 bp, Homo sapiens
tctctgacttccgcgttcaaa

SEQ ID NO: 19 - DNA, 21 bp, Homo sapiens
tcagttcaacatcacagatga

SEQ ID NO: 20 - DNA, 19 bp, Homo sapiens
tagagggacaagtgcgttc

SEQ ID NO: 21 - DNA, 27 bp, Artificial
  Synthetic oligonucleotide
cgctgaggccagtcagtcagtcagtgt

SEQ ID NO: 22 - DNA, 20 bp, Artificial
  Synthetic oligonucleotide
tgatgggaccttcttctggg

SEQ ID NO: 23 - DNA, 27 bp, Artificial
  Synthetic oligonucleotide
catccatggtgtggggaaagttcttct

SEQ ID NO: 24 - DNA, 22 bp, Artificial
  Synthetic oligonucleotide
gccattgtaataactccgcacc

SEQ ID NO: 25 - DNA, 28 bp, Artificial
  Synthetic oligonucleotide
tcagtcagtgtggggaaagttcttctgg

SEQ ID NO: 26 - RNA, 19 nt, Artificial
  Synthetic oligonucleotide
ccacuugcccagcuauagg

SEQ ID NO: 27 - RNA, 19 nt, Artificial
  Synthetic oligonucleotide
ugugcuguauagaugaucc

SEQ ID NO: 28 - DNA, 21 bp, Artificial
  Synthetic oligonucleotide
ccuauagcugggcaaguggtt

SEQ ID NO: 29 - DNA, 21 bp, Artificial
  Synthetic oligonucleotide
ccacuugcccagcuauaggtt

SEQ ID NO: 30 - DNA, 21 bp, Artificial
  Synthetic oligonucleotide
ggaucaucuauacagcacatt

SEQ ID NO: 31 - DNA, 21 bp, Artificial
  Synthetic oligonucleotide
ugugcuguauagaugaucctt